European Patent Specification EP 3 147 369 B1, published August 6, 2025. Title: Method for producing fibroin-like protein. Applicant: Ajinomoto Co., Inc. The sequence listing filed with the application follows.

SEQUENCE LISTING (5 sequences)

SEQ ID NO: 1 - DNA, 3465 bp, Artificial Sequence
  fibroin-like protein gene
  CDS (1)..(3465)
atgcatcaccatcatcatcatcaccaccaccattcctcgggctcatccttggaagtgttatttcaaggaccagcacgagccggttcgggacaacaagggcctggccagcagggcccaggtcaacaagggccaggacagcagggtccttatgggcccggcgcaagcgcagcagctgcggccgctggtggctatggtcctggctccggtcaacagggcccttcgcaacaaggtcccgggcagcaaggtcctggtggccagggtccctacgggccgggggcgagtgcggcagcagccgctgcaggcggttatggtccaggaagcggacagcaaggtccgggaggtcaaggtccgtatggcccaggctctagcgcggctgccgctgccgcgggtggcaacggaccagggagcggacaacagggcgcgggacaacagggtccaggacagcaaggcccaggggcgtcggcggctgcagcggcggccggaggctatggacccggctcaggacaacagggaccgggtcaacaaggacccggtggccaaggcccctatggcccgggcgccagcgcggccgcagccgccgcgggcgggtacggccccggtagcggccagggaccaggtcagcaggggccaggaggtcagggcccatacggtccgggcgcatccgcggcggcggcagcggcaggtggctacggtcccggaagcggccaacaggggccagggcaacaaggaccaggacaacaaggtcctgggggccaaggaccgtatggaccaggagcatcagctgcagccgcggcagctggcggttacggtccaggctacggccagcagggtccgggtcagcagggaccgggaggccaggggccttatggccctggcgcttccgcagccagtgccgcttctggaggatacgggccgggaagcggtcagcaaggccctggccaacaaggacctggaggccaagggccctacggcccaggagcctcggcagccgcagctgccgcaggtgggtatgggccaggtagcgggcaacaagggccgggtcagcaaggaccggggcaacagggacctgggcagcaaggacccgggggtcaaggcccgtacggacctggtgcgtctgcagctgctgctgcggctggtggatatggtccgggatcggggcagcagggtcccggtcagcagggccctggtcagcaagggccaggccaacagggacccggacaacaaggcccgggtcaacagggtcctggacagcaggggccgggccaacaaggccctgggcaacagggtccggggggacagggggcctatgggcctggcgcatctgccgccgctggcgcagccggtgggtacgggcctgggtcaggtcaacaggggcctggtcaacaaggccccgggcaacagggccccggccagcaaggtccagggcagcagggcccgggacagcaagggcctggacaacaggggcccggacagcagggaccttacgggcccggtgcgagcgcagcggccgccgccgcagggggatatggccccggatcgggccagcagggaccaggccagcaaggacctggccaacagggcccggggggtcaggggccgtatggtcccggcgctgcaagtgctgcagtgtccgtttctagagcacgagccggttcgggacaacaagggcctggccagcagggcccaggtcaacaagggccaggacagcagggtccttatgggcccggcgcaagcgcagcagctgcggccgctggtggctatggtcctggctccggtcaacagggcccttcgcaacaaggtcccgggcagcaaggtcctggtggccagggtccctacgggccgggggcgagtgcggcagcagccgctgcaggcggttatggtccaggaagcggacagcaaggtccgggaggtcaaggtccgtatggcccaggctctagcgcggctgccgctgccgcgggtggcaacggaccagggagcggacaacagggcgcgggacaacagggtccaggacagcaaggcccaggggcgtcggcggctgcagcggcggccggaggctatggacccggctcaggacaacagggaccgggtcaacaaggacccggtggccaaggcccctatggcccgggcgccagcgcggccgcagccgccgcgggcgggtacggccccggtagcggccagggaccaggtcagcaggggccaggaggtcagggcccatacggtccgggcgcatccgcggcggcggcagcggcaggtggctacggtcccggaagcggccaacaggggccagggcaacaaggaccaggacaacaaggtcctgggggccaaggaccgtatggaccaggagcatcagctgcagccgcggcagctggcggttacggtccaggctacggccagcagggtccgggtcagcagggaccgggaggccaggggccttatggccctggcgcttccgcagccagtgccgcttctggaggatacgggccgggaagcggtcagcaaggccctggccaacaaggacctggaggccaagggccctacggcccaggagcctcggcagccgcagctgccgcaggtgggtatgggccaggtagcgggcaacaagggccgggtcagcaaggaccggggcaacagggacctgggcagcaaggacccgggggtcaaggcccgtacggacctggtgcgtctgcagctgctgctgcggctggtggatatggtccgggatcggggcagcagggtcccggtcagcagggccctggtcagcaagggccaggccaacagggacccggacaacaaggcccgggtcaacagggtcctggacagcaggggccgggccaacaaggccctgggcaacagggtccggggggacagggggcctatgggcctggcgcatctgccgccgctggcgcagccggtgggtacgggcctgggtcaggtcaacaggggcctggtcaacaaggccccgggcaacagggccccggccagcaaggtccagggcagcagggcccgggacagcaagggcctggacaacaggggcccggacagcagggaccttacgggcccggtgcgagcgcagcggccgccgccgcagggggatatggccccggatcgggccagcagggaccaggccagcaaggacctggccaacagggcccggggggtcaggggccgtatggtcccggcgctgcaagtgctgcagtgtccgttggaggttacggccctcagtcttcgtctgttccggtggcgtccgcagttgcgagtagactgtcttcacctgctgcttcatcgcgagtatcgagcgctgtttcgtctcttgtctcgtcgggtcccacgaaacatgccgccctttcaaatacgatttcatctgtagtgtcccaagttagtgcaagtaacccggggttatccggatgcgacgttctcgttcaggcactcctagaagtagtatccgcgttggtgagcatcttataa

SEQ ID NO: 2 - protein, 1154 aa, Artificial Sequence
  Synthetic Construct
MHHHHHHHHHHSSGSSLEVLFQGPARAGSGQQGPGQQGPGQQGPGQQGPYGPGASAAAAAAGGYGPGSGQQGPSQQGPGQQGPGGQGPYGPGASAAAAAAGGYGPGSGQQGPGGQGPYGPGSSAAAAAAGGNGPGSGQQGAGQQGPGQQGPGASAAAAAAGGYGPGSGQQGPGQQGPGGQGPYGPGASAAAAAAGGYGPGSGQGPGQQGPGGQGPYGPGASAAAAAAGGYGPGSGQQGPGQQGPGQQGPGGQGPYGPGASAAAAAAGGYGPGYGQQGPGQQGPGGQGPYGPGASAASAASGGYGPGSGQQGPGQQGPGGQGPYGPGASAAAAAAGGYGPGSGQQGPGQQGPGQQGPGQQGPGGQGPYGPGASAAAAAAGGYGPGSGQQGPGQQGPGQQGPGQQGPGQQGPGQQGPGQQGPGQQGPGQQGPGGQGAYGPGASAAAGAAGGYGPGSGQQGPGQQGPGQQGPGQQGPGQQGPGQQGPGQQGPGQQGPYGPGASAAAAAAGGYGPGSGQQGPGQQGPGQQGPGGQGPYGPGAASAAVSVSRARAGSGQQGPGQQGPGQQGPGQQGPYGPGASAAAAAAGGYGPGSGQQGPSQQGPGQQGPGGQGPYGPGASAAAAAAGGYGPGSGQQGPGGQGPYGPGSSAAAAAAGGNGPGSGQQGAGQQGPGQQGPGASAAAAAAGGYGPGSGQQGPGQQGPGGQGPYGPGASAAAAAAGGYGPGSGQGPGQQGPGGQGPYGPGASAAAAAAGGYGPGSGQQGPGQQGPGQQGPGGQGPYGPGASAAAAAAGGYGPGYGQQGPGQQGPGGQGPYGPGASAASAASGGYGPGSGQQGPGQQGPGGQGPYGPGASAAAAAAGGYGPGSGQQGPGQQGPGQQGPGQQGPGGQGPYGPGASAAAAAAGGYGPGSGQQGPGQQGPGQQGPGQQGPGQQGPGQQGPGQQGPGQQGPGQQGPGGQGAYGPGASAAAGAAGGYGPGSGQQGPGQQGPGQQGPGQQGPGQQGPGQQGPGQQGPGQQGPYGPGASAAAAAAGGYGPGSGQQGPGQQGPGQQGPGGQGPYGPGAASAAVSVGGYGPQSSSVPVASAVASRLSSPAASSRVSSAVSSLVSSGPTKHAALSNTISSVVSQVSASNPGLSGCDVLVQALLEVVSALVSIL

SEQ ID NO: 3 - protein, 636 aa, Araneus diadematus
ARAGSGQQGPGQQGPGQQGPGQQGPYGPGASAAAAAAGGYGPGSGQQGPSQQGPGQQGPGGQGPYGPGASAAAAAAGGYGPGSGQQGPGGQGPYGPGSSAAAAAAGGNGPGSGQQGAGQQGPGQQGPGASAAAAAAGGYGPGSGQQGPGQQGPGGQGPYGPGASAAAAAAGGYGPGSGQGPGQQGPGGQGPYGPGASAAAAAAGGYGPGSGQQGPGQQGPGQQGPGGQGPYGPGASAAAAAAGGYGPGYGQQGPGQQGPGGQGPYGPGASAASAASGGYGPGSGQQGPGQQGPGGQGPYGPGASAAAAAAGGYGPGSGQQGPGQQGPGQQGPGQQGPGGQGPYGPGASAAAAAAGGYGPGSGQQGPGQQGPGQQGPGQQGPGQQGPGQQGPGQQGPGQQGPGQQGPGGQGAYGPGASAAAGAAGGYGPGSGQQGPGQQGPGQQGPGQQGPGQQGPGQQGPGQQGPGQQGPYGPGASAAAAAAGGYGPGSGQQGPGQQGPGQQGPGGQGPYGPGAASAAVSVGGYGPQSSSVPVASAVASRLSSPAASSRVSSAVSSLVSSGPTKHAALSNTISSVVSQVSASNPGLSGCDVLVQALLEVVSALVSILGSSSIGQINYGASAQYTQMVGQSVAQALA

SEQ ID NO: 4 - DNA, 2190 bp, Araneus diadematus
agatatacataatgcaccaccatcaccaccatcatcaccatcatagcagcggcagcagcctggaagttctgtttcagggtccggcgcgtgcgggtagcggccagcagggcccgggtcagcagggtccgggccaacaaggtccgggccagcagggcccgtatggtccgggtgcaagcgcagcagcagcggccgcaggcggttacggcccgggtagcggccagcagggcccgagccagcagggcccgggccagcagggtccgggcggtcagggtccgtacggtccgggcgcgagcgcggccgccgcggccgcaggcggttacgggccgggcagcggtcagcagggcccgggcggtcagggcccgtatggcccgggtagcagcgcggccgcggcggccgcaggcggtaatggtccgggcagcggccagcagggtgcgggccaacaaggcccgggtcagcagggcccgggtgccagcgccgccgcagcggccgcaggcggttacggtccgggtagcggtcagcagggtcctggccaacaaggcccgggcggtcaaggtccttacggcccgggcgccagcgccgcggctgcggccgcaggcggttacggaccgggtagcggccagggtcctggtcaacaaggtccgggcggtcaaggcccgtatggtccgggcgccagcgcggcggccgcggccgcaggcggttacgggccaggtagcggccagcagggtcctggccagcagggtcctggacaacaaggaccgggcggtcaaggaccgtacggcccgggcgcgagcgccgcggcagcggccgcaggcggttatggtccgggttacggtcagcagggtcccggtcaacagggaccgggcggtcaaggtccgtatggcccgggtgcgagcgcggccagcgcagcgagcggcggttacggtcctggttctggtcagcagggtcctggacagcaaggtccgggcggtcagggaccttacggtccgggtgcgagcgccgcagcggccgcagcgggcggttacggccctggctctggtcagcagggtccaggtcaacagggtcctggtcaacagggtcccggtcagcaaggcccgggcggtcagggtccttatggtccgggcgcaagcgcggccgccgccgcagcgggcggttacggtcctggcagtggtcagcagggtccgggacaacagggtcctggacagcagggtcctgggcagcagggtcctggtcagcaaggtcctggtcagcagggccctggccagcagggtcccggtcagcagggccctggtcaacaaggaccgggcggtcagggcgcgtatggtccgggtgccagcgccgcagcgggcgccgcaggcggttacgggcctggtagtggtcaacaggggcctggccaacagggccctggtcagcaaggccctggtcaacagggccctggtcagcagggccccggtcaacagggccccggtcaacagggtccaggtcagcaaggtccgtacggcccgggcgcaagcgccgcggcagcggccgcaggcggttacgggcccggctctggtcaacaggggcccggtcaacagggcccaggtcaacaggggccgggcggtcaagggccttatggcccgggcgccgcgagcgccgccgtgagcgttggcggttacggtccgcagagcagcagcgtgccggttgccagcgcagtggccagccgcctgagcagcccggccgcgagcagccgtgtgagcagcgcagttagcagcttagtgagcagcggtccgaccaaacatgccgcgctgagcaacacgattagcagcgtggttagccaggtttctgcaagcaatccgggtctgagcggttgcgatgtgctggttcaggcgctgctggaagtggttagcgccttagtgagcatcctgggcagcagcagcattggccagatcaattatggcgcgagcgcccagtacacccagatggttggtcagagcgtggcacaggccctggcgtgaaattcgagctccgtcgacaagcttgcggccgcactcgagcaccaccaccaccaccactgagatccggctgctaacaaagcccgaaaggaagctgagttggctgctgccaccgctgagcaataactagcataaccccttggggcctctaaacgggtcttgaggggttttttgctgaaaggaggaactatatccggat

SEQ ID NO: 5 - protein, 660 aa, Araneus diadematus
MHHHHHHHHHHSSGSSLEVLFQGPARAGSGQQGPGQQGPGQQGPGQQGPYGPGASAAAAAAGGYGPGSGQQGPSQQGPGQQGPGGQGPYGPGASAAAAAAGGYGPGSGQQGPGGQGPYGPGSSAAAAAAGGNGPGSGQQGAGQQGPGQQGPGASAAAAAAGGYGPGSGQQGPGQQGPGGQGPYGPGASAAAAAAGGYGPGSGQGPGQQGPGGQGPYGPGASAAAAAAGGYGPGSGQQGPGQQGPGQQGPGGQGPYGPGASAAAAAAGGYGPGYGQQGPGQQGPGGQGPYGPGASAASAASGGYGPGSGQQGPGQQGPGGQGPYGPGASAAAAAAGGYGPGSGQQGPGQQGPGQQGPGQQGPGGQGPYGPGASAAAAAAGGYGPGSGQQGPGQQGPGQQGPGQQGPGQQGPGQQGPGQQGPGQQGPGQQGPGGQGAYGPGASAAAGAAGGYGPGSGQQGPGQQGPGQQGPGQQGPGQQGPGQQGPGQQGPGQQGPYGPGASAAAAAAGGYGPGSGQQGPGQQGPGQQGPGGQGPYGPGAASAAVSVGGYGPQSSSVPVASAVASRLSSPAASSRVSSAVSSLVSSGPTKHAALSNTISSVVSQVSASNPGLSGCDVLVQALLEVVSALVSILGSSSIGQINYGASAQYTQMVGQSVAQALA